European Patent Application EP 4 610 273 A1, published September 3, 2025. Title: Novel BBD29_RS02010 variant and a method for producing L-arginine using the same. Applicant: CJ CheilJedang Corporation. The sequence listing filed with the application follows.

SEQUENCE LISTING (8 sequences)

SEQ ID NO: 1 - protein, 359 aa, synthetic construct
MTSFNKDLTLRDTAIEGLLILDFPVHGDNRGWFKENWQREKMTALGLPDFGPVQNNMSFNATAGTTRGLHAEPWDKFVSVGTGKVFGAWCDLREGSPTFGAVVTQEITPDVGVYVPRGVANGFQALEDNTLYTYLVNDHWSPNAHYANVNLDMIDWPLPITEISDKDKNHPALADASPLPSRKVLVTGARGQLGTALRAVFPTAEFVGREELDITGPLDRPWKQYSAIINAAAYTAVDKAEDEGRAAAWAINAQAVASLATVARENNLTLVHISSDYVFDGTANGEYTEDAPLSPLGVYGQTKAAGDIAASTAPRHYVVRTSWVIGDGNNFVRGWEVMPCRRRSPVFSQAVSCGSSMPR

SEQ ID NO: 2 - DNA, 1080 bp, synthetic construct
  source 1..1080: mol_type = other DNA
atgacctcattcaataaagacctcaccctgcgtgacaccgccatcgagggtctgctgattcttgatttccccgtccacggtgataaccgcggctggttcaaggagaactggcagcgggagaagatgaccgcgcttggtctgccggatttcgggccggtgcaaaacaatatgagcttcaacgcgactgccggcaccacccgtggtctgcacgccgagccctgggacaagttcgtctccgtgggcaccggcaaggtcttcggcgcgtggtgcgatctgcgtgagggatcacccacctttggtgcggtggtcacccaggaaatcaccccggatgtcggcgtctacgtcccgcgcggggtggccaacggtttccaggcgctcgaggacaacaccctttatacctacctggtcaatgatcactggtcacctaacgcgcactacgccaacgtcaacctcgacatgatcgactggcccctgccgatcaccgagatctccgacaaggacaaaaaccaccccgcgcttgccgacgcctcccccctgccctcccgcaaggttctggtcacgggcgcgcgcgggcagttgggcaccgccctgcgggcggtgttcccgacggccgaattcgtcggccgtgaggaactcgatatcacgggcccgctggatcgtccctggaagcagtactccgccatcatcaacgccgcggcctacacggcagtggataaggccgaagacgaaggtcgcgctgcagcctgggccatcaacgctcaggcggtggccagcctggccacggtggcccgggagaacaacctcaccctggtgcatatctcctccgactacgtcttcgacggcaccgccaatggtgagtacaccgaggatgcgccactatcccccttgggtgtctacggccagaccaaggccgccggtgatatcgcagcgtccaccgcacctcggcattatgtggtgcgcaccagctgggtcatcggcgatggcaacaacttcgtgcggggctgggaagttatgccgtgcaggcgacgatctccggtattctctcaggctgtcagctgtggaagcagtatgccgcgttga

SEQ ID NO: 3 - protein, 359 aa, synthetic construct
MTSFNKDLTLRDTAIEGLLILDFPVHGDNRGWFKENWQREKMTALGLPDFGPVQNNMSFNATAGTTRGLHAEPWDKFVSVGTGKVFGAWCDLREGSPTFGAVVTQEITPDVGVYVPRGVANGFQALEDNTLYTYLVNDHWSPNAHYANVNLDMIDWPLPITEISDKDKNHPALADASPLPSRKVLVTGARGQLGTALRAVFPTAEFVGREELDITGPLDRPWKQYSAIINAAAYTAVDKAEDEGRAAAWAINAQAVASLATVARENNLTLVHISSDYVFDGTANGEYTEDAPLSPLGVYGQTKAAGDIAASTAPRHYVVRTSWVIGDGNNFVRGWEVMPCRRRSPVFSRAVSCGSSMPR

SEQ ID NO: 4 - DNA, 1080 bp, synthetic construct
  source 1..1080: mol_type = other DNA
atgacctcattcaataaagacctcaccctgcgtgacaccgccatcgagggtctgctgattcttgatttccccgtccacggtgataaccgcggctggttcaaggagaactggcagcgggagaagatgaccgcgcttggtctgccggatttcgggccggtgcaaaacaatatgagcttcaacgcgactgccggcaccacccgtggtctgcacgccgagccctgggacaagttcgtctccgtgggcaccggcaaggtcttcggcgcgtggtgcgatctgcgtgagggatcacccacctttggtgcggtggtcacccaggaaatcaccccggatgtcggcgtctacgtcccgcgcggggtggccaacggtttccaggcgctcgaggacaacaccctttatacctacctggtcaatgatcactggtcacctaacgcgcactacgccaacgtcaacctcgacatgatcgactggcccctgccgatcaccgagatctccgacaaggacaaaaaccaccccgcgcttgccgacgcctcccccctgccctcccgcaaggttctggtcacgggcgcgcgcgggcagttgggcaccgccctgcgggcggtgttcccgacggccgaattcgtcggccgtgaggaactcgatatcacgggcccgctggatcgtccctggaagcagtactccgccatcatcaacgccgcggcctacacggcagtggataaggccgaagacgaaggtcgcgctgcagcctgggccatcaacgctcaggcggtggccagcctggccacggtggcccgggagaacaacctcaccctggtgcatatctcctccgactacgtcttcgacggcaccgccaatggtgagtacaccgaggatgcgccactatcccccttgggtgtctacggccagaccaaggccgccggtgatatcgcagcgtccaccgcacctcggcattatgtggtgcgcaccagctgggtcatcggcgatggcaacaacttcgtgcggggctgggaagttatgccgtgcaggcgacgatctccggtattctctcgggctgtcagctgtggaagcagtatgccgcgttga

SEQ ID NO: 5 - DNA, 38 bp, synthetic construct
  source 1..38: mol_type = other DNA
tgaattcgagctcggtaccccaaggttctggtcacggg

SEQ ID NO: 6 - DNA, 28 bp, synthetic construct
  source 1..28: mol_type = other DNA
gctgacagcctgagagaataccggagat

SEQ ID NO: 7 - DNA, 28 bp, synthetic construct
  source 1..28: mol_type = other DNA
gtattctctcaggctgtcagctgtggaa

SEQ ID NO: 8 - DNA, 38 bp, synthetic construct
  source 1..38: mol_type = other DNA
gtcgactctagaggatcccctgacggggttgagccaag